European Patent Specification EP 3 355 797 B1, published October 25, 2023. Title: Micro-needle sampling device and use thereof. Applicant: Kamerton, Kathryn Smith, Michael J. The sequence listing filed with the application follows.

SEQUENCE LISTING (3 sequences)

SEQ ID NO: 1 - DNA, 22 bp, Bos taurus
ctaagatcatggcatcaggtcc

SEQ ID NO: 2 - DNA, 21 bp, Bos taurus
ccccaaaataaagtcagccac

SEQ ID NO: 3 - DNA, 26 bp, Bos taurus
  misc_feature (1)..(1): 6-carboxyfluorescein
  misc_feature (26)..(26): tetramethylrhodamine
tccactgtttccccatctatttgcca